European Patent Application EP 4 321 172 A2, published February 14, 2024. Title: Novel peptides and combination of peptides for use in immunotherapy against esophageal cancer and other cancers. Applicant: immatics biotechnologies GmbH. The sequence listing filed with the application follows.

SEQUENCE LISTING (103 sequences)

SEQ ID NO: 1 - protein, 9 aa, Homo sapiens
STYGGGLSV

SEQ ID NO: 2 - protein, 13 aa, Homo sapiens
SLYNLGGSKRISI

SEQ ID NO: 3 - protein, 9 aa, Homo sapiens
TASAITPSV

SEQ ID NO: 4 - protein, 9 aa, Homo sapiens
ALFGTILEL

SEQ ID NO: 5 - protein, 9 aa, Homo sapiens
NLMASQPQL

SEQ ID NO: 6 - protein, 9 aa, Homo sapiens
LLSGDLIFL

SEQ ID NO: 7 - protein, 10 aa, Homo sapiens
SIFEGLLSGV

SEQ ID NO: 8 - protein, 13 aa, Homo sapiens
ALLDGGSEAYWRV

SEQ ID NO: 9 - protein, 9 aa, Homo sapiens
HLIAEIHTA

SEQ ID NO: 10 - protein, 10 aa, Homo sapiens
SLDENSDQQV

SEQ ID NO: 11 - protein, 11 aa, Homo sapiens
ALWLPTDSATV

SEQ ID NO: 12 - protein, 9 aa, Homo sapiens
GLASRILDA

SEQ ID NO: 13 - protein, 9 aa, Homo sapiens
SLSPVILGV

SEQ ID NO: 14 - protein, 9 aa, Homo sapiens
RLPNAGTQV

SEQ ID NO: 15 - protein, 9 aa, Homo sapiens
LLANGVYAA

SEQ ID NO: 16 - protein, 9 aa, Homo sapiens
VLAEGGEGV

SEQ ID NO: 17 - protein, 8 aa, Homo sapiens
MISRTPEV

SEQ ID NO: 18 - protein, 10 aa, Homo sapiens
FLLDQVQLGL

SEQ ID NO: 19 - protein, 10 aa, Homo sapiens
GLAPFLLNAV

SEQ ID NO: 20 - protein, 12 aa, Homo sapiens
IIEVDPDTKEML

SEQ ID NO: 21 - protein, 9 aa, Homo sapiens
IVREFLTAL

SEQ ID NO: 22 - protein, 9 aa, Homo sapiens
KLNDTYVNV

SEQ ID NO: 23 - protein, 9 aa, Homo sapiens
KLSDSATYL

SEQ ID NO: 24 - protein, 9 aa, Homo sapiens
LLFAGTMTV

SEQ ID NO: 25 - protein, 9 aa, Homo sapiens
LLPPPPPPA

SEQ ID NO: 26 - protein, 9 aa, Homo sapiens
MLAEKLLQA

SEQ ID NO: 27 - protein, 9 aa, Homo sapiens
NLREGDQLL

SEQ ID NO: 28 - protein, 9 aa, Homo sapiens
SLDGFTIQV

SEQ ID NO: 29 - protein, 9 aa, Homo sapiens
SLDGTELQL

SEQ ID NO: 30 - protein, 9 aa, Homo sapiens
SLNGNQVTV

SEQ ID NO: 31 - protein, 9 aa, Homo sapiens
VLPKLYVKL

SEQ ID NO: 32 - protein, 9 aa, Homo sapiens
YMLDIFHEV

SEQ ID NO: 33 - protein, 12 aa, Homo sapiens
GLDVTSLRPFDL

SEQ ID NO: 34 - protein, 10 aa, Homo sapiens
SLVSEQLEPA

SEQ ID NO: 35 - protein, 9 aa, Homo sapiens
LLRFSQDNA

SEQ ID NO: 36 - protein, 10 aa, Homo sapiens
FLLRFSQDNA

SEQ ID NO: 37 - protein, 12 aa, Homo sapiens
YTQPFSHYGQAL

SEQ ID NO: 38 - protein, 9 aa, Homo sapiens
IAAIRGFLV

SEQ ID NO: 39 - protein, 10 aa, Homo sapiens
LVRDTQSGSL

SEQ ID NO: 40 - protein, 9 aa, Homo sapiens
GLAFSLYQA

SEQ ID NO: 41 - protein, 12 aa, Homo sapiens
GLESEELEPEEL

SEQ ID NO: 42 - protein, 9 aa, Homo sapiens
TQTAVITRI

SEQ ID NO: 43 - protein, 9 aa, Homo sapiens
KVVGKDYLL

SEQ ID NO: 44 - protein, 14 aa, Homo sapiens
ATGNDRKEAAENSL

SEQ ID NO: 45 - protein, 9 aa, Homo sapiens
MLTELEKAL

SEQ ID NO: 46 - protein, 11 aa, Homo sapiens
YTAQIGADIAL

SEQ ID NO: 47 - protein, 9 aa, Homo sapiens
VLASGFLTV

SEQ ID NO: 48 - protein, 10 aa, Homo sapiens
SMHQMLDQTL

SEQ ID NO: 49 - protein, 9 aa, Homo sapiens
GLMKDIVGA

SEQ ID NO: 50 - protein, 11 aa, Homo sapiens
GMNPHQTPAQL

SEQ ID NO: 51 - protein, 9 aa, Homo sapiens
KLFGHLTSA

SEQ ID NO: 52 - protein, 12 aa, Homo sapiens
VAIGGVDGNVRL

SEQ ID NO: 53 - protein, 9 aa, Homo sapiens
VVVTGLTLV

SEQ ID NO: 54 - protein, 9 aa, Homo sapiens
YQDLLNVKM

SEQ ID NO: 55 - protein, 9 aa, Homo sapiens
GAIDLLHNV

SEQ ID NO: 56 - protein, 9 aa, Homo sapiens
ALVEVTEHV

SEQ ID NO: 57 - protein, 10 aa, Homo sapiens
GLAPNTPGKA

SEQ ID NO: 58 - protein, 9 aa, Homo sapiens
LILESIPVV

SEQ ID NO: 59 - protein, 9 aa, Homo sapiens
SLLDTLREV

SEQ ID NO: 60 - protein, 9 aa, Homo sapiens
VVMEELLKV

SEQ ID NO: 61 - protein, 9 aa, Homo sapiens
TQTTHELTI

SEQ ID NO: 62 - protein, 10 aa, Homo sapiens
ALYEYQPLQI

SEQ ID NO: 63 - protein, 10 aa, Homo sapiens
LAYTLGVKQL

SEQ ID NO: 64 - protein, 9 aa, Homo sapiens
GLTDVIRDV

SEQ ID NO: 65 - protein, 11 aa, Homo sapiens
YVVGGFLYQRL

SEQ ID NO: 66 - protein, 9 aa, Homo sapiens
LLDEKVQSV

SEQ ID NO: 67 - protein, 9 aa, Homo sapiens
SMNGGVFAV

SEQ ID NO: 68 - protein, 12 aa, Homo sapiens
PAVLQSSGLYSL

SEQ ID NO: 69 - protein, 11 aa, Homo sapiens
GLLVGSEKVTM

SEQ ID NO: 70 - protein, 9 aa, Homo sapiens
FVLDTSESV

SEQ ID NO: 71 - protein, 12 aa, Homo sapiens
ASDPILYRPVAV

SEQ ID NO: 72 - protein, 9 aa, Homo sapiens
FLPPAQVTV

SEQ ID NO: 73 - protein, 9 aa, Homo sapiens
KITEAIQYV

SEQ ID NO: 74 - protein, 9 aa, Homo sapiens
ILASLATSV

SEQ ID NO: 75 - protein, 10 aa, Homo sapiens
GLMDDVDFKA

SEQ ID NO: 76 - protein, 9 aa, Homo sapiens
KVADYIPQL

SEQ ID NO: 77 - protein, 10 aa, Homo sapiens
VLVPYEPPQV

SEQ ID NO: 78 - protein, 9 aa, Homo sapiens
KVANIIAEV

SEQ ID NO: 79 - protein, 9 aa, Homo sapiens
GQDVGRYQV

SEQ ID NO: 80 - protein, 9 aa, Homo sapiens
ALQEALENA

SEQ ID NO: 81 - protein, 9 aa, Homo sapiens
AVLPHVDQV

SEQ ID NO: 82 - protein, 9 aa, Homo sapiens
HLLGHLEQA

SEQ ID NO: 83 - protein, 10 aa, Homo sapiens
ALADGVVSQA

SEQ ID NO: 84 - protein, 9 aa, Homo sapiens
SLAESLDQA

SEQ ID NO: 85 - protein, 9 aa, Homo sapiens
NIIELVHQV

SEQ ID NO: 86 - protein, 9 aa, Homo sapiens
GLLTEIRAV

SEQ ID NO: 87 - protein, 9 aa, Homo sapiens
FLDNGPKTI

SEQ ID NO: 88 - protein, 9 aa, Homo sapiens
GLWEQENHL

SEQ ID NO: 89 - protein, 9 aa, Homo sapiens
SLADSLYNL

SEQ ID NO: 90 - protein, 9 aa, Homo sapiens
SIYEYYHAL

SEQ ID NO: 91 - protein, 9 aa, Homo sapiens
KLIDDVHRL

SEQ ID NO: 92 - protein, 9 aa, Homo sapiens
SILRHVAEV

SEQ ID NO: 93 - protein, 9 aa, Homo sapiens
VLINTSVTL

SEQ ID NO: 94 - protein, 11 aa, Homo sapiens
TLLQEQGTKTV

SEQ ID NO: 95 - protein, 9 aa, Homo sapiens
LIQDRVAEV

SEQ ID NO: 96 - protein, 10 aa, Homo sapiens
GAAVRIGSVL

SEQ ID NO: 97 - protein, 9 aa, Homo sapiens
ELDRTPPEV

SEQ ID NO: 98 - protein, 9 aa, Homo sapiens
VLFPNLKTV

SEQ ID NO: 99 - protein, 10 aa, Homo sapiens
RVAPEEHPVL

SEQ ID NO: 100 - protein, 10 aa, Homo sapiens
GLYPDAFAPV

SEQ ID NO: 101 - protein, 9 aa, Homo sapiens
AMTQLLAGV

SEQ ID NO: 102 - protein, 10 aa, Homo sapiens
ELAGIGILTV

SEQ ID NO: 103 - protein, 9 aa, Homo sapiens
YLLPAIVHI